European Patent Application EP 4 299 728 A1, published January 3, 2024. Title: RECOMBINANT SPRIVIVIRUSES, USES THEREOF AND METHODS FOR PRODUCING THE SAME. Applicant: Institut national de recherche pour l'agriculture, l'alimentation et l'environnement Université de Versailles Saint-Quentin en Yvelines Universidade de Santiago de Compostela. The sequence listing filed with the application follows.

SEQUENCE LISTING (16 sequences)

SEQ ID NO: 1 - RNA, 13 nt, Spring viremia of carp virus
uugucucuaguac

SEQ ID NO: 2 - RNA, 13 nt, Spring viremia of carp virus
uugucuguaguac

SEQ ID NO: 3 - RNA, 11 nt, Spring viremia of carp virus
auacuuuuuuu

SEQ ID NO: 4 - protein, 8 aa, Artificial Sequence
  consensus sequence of 2A-like sequence
  misc_feature (2)..(2): X = any amino acid
  misc_feature (4)..(4): X = any amino acid
DXEXNPGP

SEQ ID NO: 5 - protein, 19 aa, Artificial Sequence
  2A-like sequence
ATNFSLLKQAGDVEENPGP

SEQ ID NO: 6 - protein, 18 aa, Artificial Sequence
  2A-like sequence
EGRGSLLTCGDVEENPGP

SEQ ID NO: 7 - protein, 20 aa, Artificial Sequence
  2A-like sequence
QCTNYALLKLAGDVESNPGP

SEQ ID NO: 8 - protein, 22 aa, Artificial Sequence
  2A-like sequence
VKQTLNFDLLKLAGDVESNPGP

SEQ ID NO: 9 - protein, 21 aa, Spring viremia of carp virus
MSIISYIAFLLLIDSNLGIPI

SEQ ID NO: 10 - protein, 42 aa, Spring viremia of carp virus
FGMTLVALILIFLLIRCCVACTYLMKRSKRPATESHEMRSLV

SEQ ID NO: 11 - protein, 34 aa, Spring viremia of carp virus
IREDDIFFDNTGENGNPVDAVVEWVSGWGTSLKF

SEQ ID NO: 12 - DNA, 30 bp, Artificial Sequence
  Consensus sequence of untranslated region from Spring viraemia of carp virus
dddrtatgaaaaaaactaacagasatcatg

SEQ ID NO: 13 - DNA, 11 bp, Spring viremia of carp virus
tatgaaaaaaa

SEQ ID NO: 14 - DNA, 13 bp, Spring viremia of carp virus
aacagasatcatg

SEQ ID NO: 15 - protein, 19 aa, Spring viremia of carp virus
MSIISYIAFLLLIDSNLGI

SEQ ID NO: 16 - DNA, 54 bp, Infectious hematopoietic necrosis virus
atggacaccacgatcaccactccgctcattctcattctgatcacctgcggagca